European Patent Specification EP 3 741 839 B1, published March 20, 2024. Title: REACTION TREATMENT DEVICE. Applicant: NIPPON SHEET GLASS COMPANY, LIMITED. The sequence listing filed with the application follows.

SEQUENCE LISTING (3 sequences)

SEQ ID NO: 1 - DNA, 25 bp, Artificial Sequence
  Forward PCR Primer
ggataatttgtttgcagttgatgtc

SEQ ID NO: 2 - DNA, 29 bp, Artificial Sequence
  Reverse PCR Primer
caaatcctgtcacatataaattatttcgt

SEQ ID NO: 3 - DNA, 31 bp, Artificial Sequence
  Probe
ccgtagattattaaaccgcccttcctctgga